European Patent Specification EP 3 436 598 B1, published January 8, 2025. Title: Method for predicting the response of melanoma patients to a medicament. Applicant: PamGene B.V. Leiden University Medical Centre. The sequence listing filed with the application follows.

SEQUENCE LISTING (189 sequences)

SEQ ID NO: 1 - protein, 13 aa, Artificial Sequence
  CDK7_157_169
GLAKSFGSPNRAY

SEQ ID NO: 2 - protein, 13 aa, Artificial Sequence
  TYRO3_679_691
KIYSGDYYRQGCA

SEQ ID NO: 3 - protein, 13 aa, Artificial Sequence
  PDPK1_369_381
EQRMKESSFYSLC

SEQ ID NO: 4 - protein, 13 aa, Artificial Sequence
  VGFR1_1326_1338
DEDCYGNYDNLLS

SEQ ID NO: 5 - protein, 13 aa, -
DYNSVVLYSTPPI

SEQ ID NO: 6 - protein, 13 aa, Artificial Sequence
  FGFR1_761_773
TSNQEYLDLSMPL

SEQ ID NO: 7 - protein, 13 aa, Artificial Sequence
  K2C6B_53_65
GAGFGSRSLYGLG

SEQ ID NO: 8 - protein, 13 aa, Artificial Sequence
  PRRX2_202_214
WTASSPYSTVPPY

SEQ ID NO: 9 - protein, 13 aa, Artificial Sequence
  VGFR3_1061_1073
DIYKDPDYVRKGS

SEQ ID NO: 10 - protein, 13 aa, Artificial Sequence
  PGFRB_709_721
RPPSAELYSNALP

SEQ ID NO: 11 - protein, 13 aa, Artificial Sequence
  FGFR2_762_774
TLTTNEEYLDLSQ

SEQ ID NO: 12 - protein, 13 aa, Artificial Sequence
  EGFR_1165_1177
ISLDNPDYQQDFF

SEQ ID NO: 13 - protein, 13 aa, Artificial Sequence
  VGFR1_1320_1332_C1320S/C1321S
SSSPPPDYNSVVL

SEQ ID NO: 14 - protein, 13 aa, Artificial Sequence
  RON_1353_1365
YVQLPATYMNLGP

SEQ ID NO: 15 - protein, 13 aa, Artificial Sequence
  PGFRB_768_780
SSNYMAPYDNYVP

SEQ ID NO: 16 - protein, 13 aa, Artificial Sequence
  RET_1022_1034
TPSDSLIYDDGLS

SEQ ID NO: 17 - protein, 13 aa, Artificial Sequence
  ANXA1_14_26
IENEEQEYVQTVK

SEQ ID NO: 18 - protein, 13 aa, Artificial Sequence
  FGFR3_753_765
TVTSTDEYLDLSA

SEQ ID NO: 19 - protein, 13 aa, Artificial Sequence
  ODBA_340_352
DDSSAYRSVDEVN

SEQ ID NO: 20 - protein, 13 aa, Artificial Sequence
  PDPK1_2_14
ARTTSQLYDAVPI

SEQ ID NO: 21 - protein, 13 aa, Artificial Sequence
  TEC_512_524
RYFLDDQYTSSSG

SEQ ID NO: 22 - protein, 13 aa, Artificial Sequence
  FER_707_719
RQEDGGVYSSSGL

SEQ ID NO: 23 - protein, 13 aa, Artificial Sequence
  PGFRB_1002_1014
LDTSSVLYTAVQP

SEQ ID NO: 24 - protein, 13 aa, Artificial Sequence
  CBL_693_705
EGEEDTEYMTPSS

SEQ ID NO: 25 - protein, 13 aa, Artificial Sequence
  RB_804_816
IYISPLKSPYKIS

SEQ ID NO: 26 - protein, 13 aa, Artificial Sequence
  VGFR2_1052_1064
DIYKDPDYVRKGD

SEQ ID NO: 27 - protein, 13 aa, Artificial Sequence
  FAK1_569_581
RYMEDSTYYKASK

SEQ ID NO: 28 - protein, 13 aa, Artificial Sequence
  MET_1227_1239
RDMYDKEYYSVHN

SEQ ID NO: 29 - protein, 13 aa, Artificial Sequence
  NTRK2_696_708
GMSRDVYSTDYYR

SEQ ID NO: 30 - protein, 13 aa, Artificial Sequence
  DYR1A_312_324
CQLGQRIYQYIQS

SEQ ID NO: 31 - protein, 13 aa, Artificial Sequence
  CD3Z_146_158
STATKDTYDALHM

SEQ ID NO: 32 - protein, 13 aa, Artificial Sequence
  DCX_109_121
GIVYAVSSDRFRS

SEQ ID NO: 33 - protein, 13 aa, Artificial Sequence
  PGFRB_771_783
YMAPYDNYVPSAP

SEQ ID NO: 34 - protein, 13 aa, Artificial Sequence
  LCK_387_399
RLIEDNEYTAREG

SEQ ID NO: 35 - protein, 13 aa, Artificial Sequence
  JAK1_1015_1027
AIETDKEYYTVKD

SEQ ID NO: 36 - protein, 13 aa, Artificial Sequence
  VGFR2_1168_1180
AQQDGKDYIVLPI

SEQ ID NO: 37 - protein, 13 aa, Artificial Sequence
  MK07_211_223
AEHQYFMTEYVAT

SEQ ID NO: 38 - protein, 13 aa, Artificial Sequence
  MBP_198_210
ARTAHYGSLPQKS

SEQ ID NO: 39 - protein, 13 aa, Artificial Sequence
  B3AT_39_51
TEATATDYHTTSH

SEQ ID NO: 40 - protein, 13 aa, Artificial Sequence
  CD3Z_116_128
KDKMAEAYSEIGM

SEQ ID NO: 41 - protein, 13 aa, Artificial Sequence
  ANXA2_17_29
HSTPPSAYGSVKA

SEQ ID NO: 42 - protein, 13 aa, Artificial Sequence
  EGFR_1190_1202
STAENAEYLRVAP

SEQ ID NO: 43 - protein, 13 aa, Artificial Sequence
  CALM_95_107
KDGNGYISAAELR

SEQ ID NO: 44 - protein, 13 aa, Artificial Sequence
  PECA1_706_718
KKDTETVYSEVRK

SEQ ID NO: 45 - protein, 13 aa, Artificial Sequence
  EPOR_361_373
SEHAQDTYLVLDK

SEQ ID NO: 46 - protein, 13 aa, Artificial Sequence
  EPHA2_765_777
EDDPEATYTTSGG

SEQ ID NO: 47 - protein, 13 aa, Artificial Sequence
  STAT4_714_726
PSDLLPMSPSVYA

SEQ ID NO: 48 - protein, 13 aa, Artificial Sequence
  FES_706_718
REEADGVYAASGG

SEQ ID NO: 49 - protein, 13 aa, Artificial Sequence
  EPHB1_771_783
DDTSDPTYTSSLG

SEQ ID NO: 50 - protein, 13 aa, Artificial Sequence
  PP2AB_297_309
EPHVTRRTPDYFL

SEQ ID NO: 51 - protein, 13 aa, Artificial Sequence
  CRK_214_226
GPPEPGPYAQPSV

SEQ ID NO: 52 - protein, 13 aa, Artificial Sequence
  LAT_249_261
EEGAPDYENLQEL

SEQ ID NO: 53 - protein, 13 aa, Artificial Sequence
  VGFR2_989_1001
EEAPEDLYKDFLT

SEQ ID NO: 54 - protein, 13 aa, Artificial Sequence
  FAK2_572_584
RYIEDEDYYKASV

SEQ ID NO: 55 - protein, 13 aa, Artificial Sequence
  CDK2_8_20
EKIGEGTYGVVYK

SEQ ID NO: 56 - protein, 13 aa, Artificial Sequence
  CTNB1_79_91
VADIDGQYAMTRA

SEQ ID NO: 57 - protein, 13 aa, Artificial Sequence
  ERBB2_1241_1253
PTAENPEYLGLDV

SEQ ID NO: 58 - protein, 13 aa, Artificial Sequence
  RON_1346_1358
SALLGDHYVQLPA

SEQ ID NO: 59 - protein, 15 aa, Artificial Sequence
  PGFRB_1014_1028
PNEGDNDYIIPLPDP

SEQ ID NO: 60 - protein, 13 aa, Artificial Sequence
  EPHA1_774_786
LDDFDGTYETQGG

SEQ ID NO: 61 - protein, 13 aa, Artificial Sequence
  ZAP70_485_497
ALGADDSYYTARS

SEQ ID NO: 62 - protein, 13 aa, Artificial Sequence
  ERBB4_1181_1193
QALDNPEYHNASN

SEQ ID NO: 63 - protein, 13 aa, Artificial Sequence
  41_654_666
LDGENIYIRHSNL

SEQ ID NO: 64 - protein, 13 aa, Artificial Sequence
  MK01_180_192
HTGFLTEYVATRW

SEQ ID NO: 65 - protein, 13 aa, Artificial Sequence
  VGFR2_1046_1058
DFGLARDIYKDPD

SEQ ID NO: 66 - protein, 13 aa, Artificial Sequence
  PAXI_24_36
FLSEETPYSYPTG

SEQ ID NO: 67 - protein, 13 aa, Artificial Sequence
  RAF1_332_344
PRGQRDSSYYWEI

SEQ ID NO: 68 - protein, 13 aa, Artificial Sequence
  ACHD_383_395
YISKAEEYFLLKS

SEQ ID NO: 69 - protein, 13 aa, Artificial Sequence
  FRK_380_392
KVDNEDIYESRHE

SEQ ID NO: 70 - protein, 13 aa, Artificial Sequence
  KSYK_518_530
ALRADENYYKAQT

SEQ ID NO: 71 - protein, 13 aa, Artificial Sequence
  RASA1_453_465
TVDGKEIYNTIRR

SEQ ID NO: 72 - protein, 13 aa, Artificial Sequence
  PLCG1_764_776
IGTAEPDYGALYE

SEQ ID NO: 73 - protein, 13 aa, Artificial Sequence
  K2C8_425_437
SAYGGLTSPGLSY

SEQ ID NO: 74 - protein, 12 aa, Artificial Sequence
  ART_004_EAIYAAPFAKKKXC
EAIYAAPFAKKK

SEQ ID NO: 75 - protein, 13 aa, Artificial Sequence
  EPOR_419_431
ASAASFEYTILDP

SEQ ID NO: 76 - protein, 13 aa, Artificial Sequence
  EGFR_1103_1115
GSVQNPVYHNQPL

SEQ ID NO: 77 - protein, 15 aa, Artificial Sequence
  JAK2_563_577
VRREVGDYGQLHETE

SEQ ID NO: 78 - protein, 13 aa, Artificial Sequence
  MK10_216_228
TSFMMTPYVVTRY

SEQ ID NO: 79 - protein, 13 aa, Artificial Sequence
  DYR1A_212_224
KHDTEMKYYIVHL

SEQ ID NO: 80 - protein, 13 aa, Artificial Sequence
  P85A_600_612
NENTEDQYSLVED

SEQ ID NO: 81 - protein, 13 aa, Artificial Sequence
  PAXI_111_123
VGEEEHVYSFPNK

SEQ ID NO: 82 - protein, 13 aa, Artificial Sequence
  EPHB4_583_595
IGHGTKVYIDPFT

SEQ ID NO: 83 - protein, 13 aa, Artificial Sequence
  MK12_178_190
ADSEMTGYVVTRW

SEQ ID NO: 84 - protein, 13 aa, Artificial Sequence
  VGFR1_1040_1052
DFGLARDIYKNPD

SEQ ID NO: 85 - protein, 13 aa, Artificial Sequence
  PGFRB_572_584
VSSDGHEYIYVDP

SEQ ID NO: 86 - protein, 13 aa, Artificial Sequence
  EPHA7_607_619
TYIDPETYEDPNR

SEQ ID NO: 87 - protein, 13 aa, Artificial Sequence
  ERBB2_870_882
LDIDETEYHADGG

SEQ ID NO: 88 - protein, 13 aa, Artificial Sequence
  LAT_194_206
MESIDDYVNVPES

SEQ ID NO: 89 - protein, 13 aa, Artificial Sequence
  VINC_815_827
KSFLDSGYRILGA

SEQ ID NO: 90 - protein, 13 aa, Artificial Sequence
  NCF1_313_325
QRSRKRLSQDAYR

SEQ ID NO: 91 - protein, 13 aa, Artificial Sequence
  ERBB4_1277_1289
IVAENPEYLSEFS

SEQ ID NO: 92 - protein, 13 aa, Artificial Sequence
  VGFR2_944_956
RFRQGKDYVGAIP

SEQ ID NO: 93 - protein, 13 aa, Artificial Sequence
  NPT2A_501_513
AKALGKRTAKYRW

SEQ ID NO: 94 - protein, 13 aa, Artificial Sequence
  C1R_199_211
TEASGYISSLEYP

SEQ ID NO: 95 - protein, 13 aa, Artificial Sequence
  FABPH_13_25
DSKNFDDYMKSLG

SEQ ID NO: 96 - protein, 13 aa, Artificial Sequence
  STAT1_694_706
DGPKGTGYIKTEL

SEQ ID NO: 97 - protein, 13 aa, Artificial Sequence
  EPHA4_589_601
LNQGVRTYVDPFT

SEQ ID NO: 98 - protein, 13 aa, Artificial Sequence
  VGFR1_1046_1058_Y1048F
DIFKNPDYVRKGD

SEQ ID NO: 99 - protein, 13 aa, Artificial Sequence
  INSR_992_1004
YASSNPEYLSASD

SEQ ID NO: 100 - protein, 13 aa, Artificial Sequence
  NTRK2_509_521
PVIENPQYFGITN

SEQ ID NO: 101 - protein, 13 aa, Artificial Sequence
  MBP_259_271
FGYGGRASDYKSA

SEQ ID NO: 102 - protein, 13 aa, Artificial Sequence
  STA5A_687_699
LAKAVDGYVKPQI

SEQ ID NO: 103 - protein, 13 aa, Artificial Sequence
  NTRK1_489_501
HIIENPQYFSDAC

SEQ ID NO: 104 - protein, 13 aa, Artificial Sequence
  PTN11_539_551
SKRKGHEYTNIKY

SEQ ID NO: 105 - protein, 13 aa, Artificial Sequence
  PLCG1_776_788
EGRNPGFYVEANP

SEQ ID NO: 106 - protein, 13 aa, Artificial Sequence
  MK14_173_185
RHTDDEMTGYVAT

SEQ ID NO: 107 - protein, 13 aa, Artificial Sequence
  MBP_263_275
GRASDYKSAHKGF

SEQ ID NO: 108 - protein, 13 aa, Artificial Sequence
  RBL2_99_111
VPTVSKGTVEGNY

SEQ ID NO: 109 - protein, 13 aa, Artificial Sequence
  RET_680_692
AQAFPVSYSSSGA

SEQ ID NO: 110 - protein, 13 aa, Artificial Sequence
  EGFR_862_874
LGAEEKEYHAEGG

SEQ ID NO: 111 - protein, 13 aa, Artificial Sequence
  INSR_1348_1360
SLGFKRSYEEHIP

SEQ ID NO: 112 - protein, 13 aa, Artificial Sequence
  PRGR_545_557
LRPDSEASQSPQY

SEQ ID NO: 113 - protein, 13 aa, Artificial Sequence
  SRC8_CHICK_470_482
VSQREAEYEPETV

SEQ ID NO: 114 - protein, 13 aa, Artificial Sequence
  EPHA2_581_593
QLKPLKTYVDPHT

SEQ ID NO: 115 - protein, 13 aa, Artificial Sequence
  VGFR1_1162_1174
VQQDGKDYIPINA

SEQ ID NO: 116 - protein, 13 aa, Artificial Sequence
  MK01_198_210
IMLNSKGYTKSID

SEQ ID NO: 117 - protein, 13 aa, Artificial Sequence
  STAT6_634_646
MGKDGRGYVPATI

SEQ ID NO: 118 - protein, 13 aa, Artificial Sequence
  VGFR2_1207_1219_C1208S
VSDPKFHYDNTAG

SEQ ID NO: 119 - protein, 13 aa, Artificial Sequence
  ZBT16_621_633
LRTHNGASPYQCT

SEQ ID NO: 120 - protein, 13 aa, Artificial Sequence
  EGFR_1118_1130
APSRDPHYQDPHS

SEQ ID NO: 121 - protein, 13 aa, Artificial Sequence
  AMPE_5_17
EREGSKRYCIQTK

SEQ ID NO: 122 - protein, 13 aa, Artificial Sequence
  FGFR3_641_653
DVHNLDYYKKTTN

SEQ ID NO: 123 - protein, 13 aa, Artificial Sequence
  VGFR1_1206_1218
GSSDDVRYVNAFK

SEQ ID NO: 124 - protein, 13 aa, Artificial Sequence
  EFS_246_258_Y253F
GGTDEGIFDVPLL

SEQ ID NO: 125 - protein, 13 aa, Artificial Sequence
  ODPAT_291_303
SMSDPGVSYRTRE

SEQ ID NO: 126 - protein, 13 aa, Artificial Sequence
  STAT4_686_698
TERGDKGYVPSVF

SEQ ID NO: 127 - protein, 13 aa, Artificial Sequence
  PLCG1_1246_1258
EGSFESRYQQPFE

SEQ ID NO: 128 - protein, 13 aa, Artificial Sequence
  TNNT1_2_14
SDTEEQEYEEEQP

SEQ ID NO: 129 - protein, 13 aa, Artificial Sequence
  EGFR_908_920
MTFGSKPYDGIPA

SEQ ID NO: 130 - protein, 13 aa, Artificial Sequence
  EPHB1_921_933
SAIKMVQYRDSFL

SEQ ID NO: 131 - protein, 13 aa, Artificial Sequence
  VGFR1_1235_1247
ATSMFDDYQGDSS

SEQ ID NO: 132 - protein, 13 aa, Artificial Sequence
  STAT3_698_710
DPGSAAPYLKTKF

SEQ ID NO: 133 - protein, 13 aa, Artificial Sequence
  CALM_93_105
FDKDGNGYISAAE

SEQ ID NO: 134 - protein, 13 aa, Artificial Sequence
  DDR1_506_518
LLLSNPAYRLLLA

SEQ ID NO: 135 - protein, 13 aa, Artificial Sequence
  EGFR_1062_1074
EDSFLQRYSSDPT

SEQ ID NO: 136 - protein, 13 aa, -
QAIKMDRYKDNFT

SEQ ID NO: 137 - protein, 13 aa, Artificial Sequence
  PERI_458_470
QRSELDKSSAHSY

SEQ ID NO: 138 - protein, 13 aa, Artificial Sequence
  VGFR1_1049_1061
KNPDYVRKGDTRL

SEQ ID NO: 139 - protein, 10 aa, Artificial Sequence
  RET_1024_1033_Y1029npY
  MOD_RES (6)..(6): 3-NO2-phosphotyrosine
SDSLIYDDGL

SEQ ID NO: 140 - protein, 10 aa, Artificial Sequence
  RET_682_691_Y687npY
  MOD_RES (6)..(6): 3-NO2-phosphotyrosine
AFPVSYSSSG

SEQ ID NO: 141 - protein, 10 aa, Artificial Sequence
  FRK_382_391_Y387npY
  MOD_RES (6)..(6): 3-NO2-phosphotyrosine
DNEDIYESRH

SEQ ID NO: 142 - protein, 10 aa, Artificial Sequence
  MK01_182_191_Y187npY
  MOD_RES (6)..(6): 3-NO2-phosphotyrosine
FGLTEYVATR

SEQ ID NO: 143 - protein, 10 aa, Artificial Sequence
  MK01_198_207_Y203npY
  MOD_RES (6)..(6): 3-NO2-phosphotyrosine
LNSKGYTKSI

SEQ ID NO: 144 - protein, 10 aa, Artificial Sequence
  CBL_695_704_Y700npY
  MOD_RES (6)..(6): 3-NO2-phosphotyrosine
EEDTEYBTPS

SEQ ID NO: 145 - protein, 10 aa, Artificial Sequence
  P85A_602_611_Y607npY
  MOD_RES (6)..(6): 3-NO2-phosphotyrosine
NTEDQYSLVE

SEQ ID NO: 146 - protein, 10 aa, Artificial Sequence
  FAK1_572_581_Y577npY
  MOD_RES (6)..(6): 3-NO2-phosphotyrosine
EDSTYYKASK

SEQ ID NO: 147 - protein, 10 aa, Artificial Sequence
  FAK1_572_581_Y576npY
  MOD_RES (5)..(5): 3-NO2-phosphotyrosine
EDSTYYKASK

SEQ ID NO: 148 - protein, 11 aa, Artificial Sequence
  CRK_216_226_Y221npY
  MOD_RES (6)..(6): 3-NO2-phosphotyrosine
PEPGPYAQPSV

SEQ ID NO: 149 - protein, 11 aa, Artificial Sequence
  MET_1229_1239_Y1235npY
  MOD_RES (7)..(7): 3-NO2-phosphotyrosine
BYDKEYYSVHN

SEQ ID NO: 150 - protein, 11 aa, Artificial Sequence
  MET_1229_1239_Y1234npY
  MOD_RES (6)..(6): 3-NO2-phosphotyrosine
BYDKEYYSVHN

SEQ ID NO: 151 - protein, 10 aa, Artificial Sequence
  PGFRB_1016_1025_Y1021npY
  MOD_RES (6)..(6): 3-NO2-phosphotyrosine
EGDNDYIIPL

SEQ ID NO: 152 - protein, 10 aa, Artificial Sequence
  MK12_180_189_Y185npY
  MOD_RES (6)..(6): 3-NO2-phosphotyrosine
SEBTGYVVTR

SEQ ID NO: 153 - protein, 10 aa, Artificial Sequence
  MBP_198_207_Y203npY
  MOD_RES (6)..(6): 3-NO2-phosphotyrosine
ARTAHYGSLP

SEQ ID NO: 154 - protein, 10 aa, Artificial Sequence
  MBP_263_272_Y268npY
  MOD_RES (6)..(6): 3-NO2-phosphotyrosine
GRASDYKSAH

SEQ ID NO: 155 - protein, 10 aa, Artificial Sequence
  CADH2_780_789_Y785npY
  MOD_RES (6)..(6): 3-NO2-phosphotyrosine
EEDQDYDLSQ

SEQ ID NO: 156 - protein, 10 aa, Artificial Sequence
  PDPK1_4_13_Y9npY
  MOD_RES (6)..(6): 3-NO2-phosphotyrosine
TTSQLYDAVP

SEQ ID NO: 157 - protein, 10 aa, Artificial Sequence
  ZAP70_287_296_Y292npY
  MOD_RES (6)..(6): 3-NO2-phosphotyrosine
LNSDGYTPEP

SEQ ID NO: 158 - protein, 10 aa, Artificial Sequence
  PGFRB_746_755_Y751npY
  MOD_RES (6)..(6): 3-NO2-phosphotyrosine
DESVDYVPBL

SEQ ID NO: 159 - protein, 10 aa, Artificial Sequence
  GHR_591_600_Y595npY
  MOD_RES (5)..(5): 3-NO2-phosphotyrosine
PVPDYTSIHI

SEQ ID NO: 160 - protein, 10 aa, Artificial Sequence
  CSK_179_188_Y184npY
  MOD_RES (6)..(6): 3-NO2-phosphotyrosine
AQDEFYRSGW

SEQ ID NO: 161 - protein, 10 aa, Artificial Sequence
  SIGLEC2_817_826_Y822npY
  MOD_RES (6)..(6): 3-NO2-phosphotyrosine
DEGIHYSELI

SEQ ID NO: 162 - protein, 9 aa, Artificial Sequence
  STAT3_701_709_Y705npY
  MOD_RES (5)..(5): 3-NO2-phosphotyrosine
SAAPYLKTK

SEQ ID NO: 163 - protein, 10 aa, Artificial Sequence
  JAK2_1002_1011_Y1007npY
  MOD_RES (6)..(6): 3-NO2-phosphotyrosine
PQDKEYYKVK

SEQ ID NO: 164 - protein, 11 aa, Artificial Sequence
  LCK_389_399_Y394npY
  MOD_RES (6)..(6): 3-NO2-phosphotyrosine
IEDNEYTAREG

SEQ ID NO: 165 - protein, 11 aa, Artificial Sequence
  INSR_994_1004_Y999npY
  MOD_RES (6)..(6): 3-NO2-phosphotyrosine
SSNPEYLSASD

SEQ ID NO: 166 - protein, 11 aa, Artificial Sequence
  INSR_1350_1360_Y1355npY
  MOD_RES (6)..(6): 3-NO2-phosphotyrosine
GFKRSYEEHIP

SEQ ID NO: 167 - protein, 11 aa, Artificial Sequence
  EGFR_1192_1202_Y1197npY
  MOD_RES (6)..(6): 3-NO2-phosphotyrosine
AENAEYLRVAP

SEQ ID NO: 168 - protein, 11 aa, Artificial Sequence
  EGFR_1011_1021_Y1016npY
  MOD_RES (6)..(6): 3-NO2-phosphotyrosine
VDADEYLIPQQ

SEQ ID NO: 169 - protein, 11 aa, Artificial Sequence
  VGFR1_1208_1218_1213npY
  MOD_RES (6)..(6): 3-NO2-phosphotyrosine
SDDVRYVNAFK

SEQ ID NO: 170 - protein, 11 aa, Artificial Sequence
  STA5A_689_699_Y694npY
  MOD_RES (6)..(6): 3-NO2-phosphotyrosine
KAVDGYVKPQI

SEQ ID NO: 171 - protein, 11 aa, Artificial Sequence
  EGFR_1064_1074_Y1069npY
  MOD_RES (6)..(6): 3-NO2-phosphotyrosine
SFLQRYSSDPT

SEQ ID NO: 172 - protein, 11 aa, Artificial Sequence
  ALK_1073_1083_Y1078npY
  MOD_RES (6)..(6): 3-NO2-phosphotyrosine
LQSPEYKLSKL

SEQ ID NO: 173 - protein, 11 aa, Artificial Sequence
  TEC_514_524_Y519npY
  MOD_RES (6)..(6): 3-NO2-phosphotyrosine
FLDDQYTSSSG

SEQ ID NO: 174 - protein, 11 aa, Artificial Sequence
  CDK2_10_20_Y15npY
  MOD_RES (6)..(6): 3-NO2-phosphotyrosine
IGEGTYGVVYK

SEQ ID NO: 175 - protein, 11 aa, Artificial Sequence
  RAF1_335_345_Y340npY
  MOD_RES (6)..(6): 3-NO2-phosphotyrosine
QRDSSYYWEIE

SEQ ID NO: 176 - protein, 11 aa, Artificial Sequence
  PECA1_708_718_Y713npY
  MOD_RES (6)..(6): 3-NO2-phosphotyrosine
DTETVYSEVRK

SEQ ID NO: 177 - protein, 11 aa, Artificial Sequence
  STAT1_696_706_Y701npY
  MOD_RES (6)..(6): 3-NO2-phosphotyrosine
PKGTGYIKTEL

SEQ ID NO: 178 - protein, 11 aa, Artificial Sequence
  ERBB2_1243_1253_Y1248npY
  MOD_RES (6)..(6): 3-NO2-phosphotyrosine
AENPEYLGLDV

SEQ ID NO: 179 - protein, 11 aa, Artificial Sequence
  PAXI_113_123_Y118npY
  MOD_RES (6)..(6): 3-NO2-phosphotyrosine
EEEHVYSFPNK

SEQ ID NO: 180 - protein, 10 aa, Artificial Sequence
  EPOR_421_430_Y426npY
  MOD_RES (6)..(6): 3-NO2-phosphotyrosine
AASFEYTILD

SEQ ID NO: 181 - protein, 11 aa, Artificial Sequence
  CTNNB1_81_91_Y86npY
  MOD_RES (6)..(6): 3-NO2-phosphotyrosine
DIDGQYABTRA

SEQ ID NO: 182 - protein, 12 aa, Artificial Sequence
  ART_003_Y4pY
  MOD_RES (4)..(4): 3-NO2-phosphotyrosine
EAIYAAPFAKKK

SEQ ID NO: 183 - protein, 11 aa, Artificial Sequence
  TIE1_1002_1012_Y1007npY
  MOD_RES (6)..(6): 3-NO2-phosphotyrosine
RGEEVYVKKTB

SEQ ID NO: 184 - protein, 11 aa, Artificial Sequence
  SELE_598_608_Y603npY
  MOD_RES (6)..(6): 3-NO2-phosphotyrosine
ESDGSYQKPSY

SEQ ID NO: 185 - protein, 11 aa, Artificial Sequence
  BCR_172_182_Y177npY
  MOD_RES (6)..(6): 3-NO2-phosphotyrosine
AEKPFYVNVEF

SEQ ID NO: 186 - protein, 9 aa, Artificial Sequence
  STAT3_701_709_Y705nY
  MOD_RES (5)..(5): 3-NO2-phosphotyrosine
SAAPYLKTK

SEQ ID NO: 187 - protein, 13 aa, Artificial Sequence
  ENOG_37_49
SGASTGIYEALEL

SEQ ID NO: 188 - protein, 13 aa, Artificial Sequence
  SRC8_CHICK_476_488
EYEPETVYEVAGA

SEQ ID NO: 189 - protein, 13 aa, Artificial Sequence
  SRC8_CHICK_492_504
YQAEENTYDEYEN